European Patent Application EP 4 379 383 A1, published June 5, 2024. Title: Biomolecule Analysis by Fluorescence Intermittence Signal Recognition. Applicant: Universität Zürich. The sequence listing filed with the application follows.

SEQUENCE LISTING (10 sequences)

SEQ ID NO: 1 - protein, 5 aa, synthetic construct
  MOD_RES 3: note = Pent-4-ynoyl
  MOD_RES 3: note = HMSiR
DDCDD

SEQ ID NO: 2 - protein, 5 aa, synthetic construct
  MOD_RES 3: note = Pent-4-ynoyl
  MOD_RES 3: note = HMSiR
DLCDD

SEQ ID NO: 3 - protein, 5 aa, synthetic construct
  MOD_RES 3: note = Pent-4-ynoyl
  MOD_RES 3: note = HMSiR
DLCLD

SEQ ID NO: 4 - protein, 5 aa, synthetic construct
  MOD_RES 3: note = Pent-4-ynoyl
  MOD_RES 3: note = HMSiR
LLCDD

SEQ ID NO: 5 - protein, 6 aa, synthetic construct
  MOD_RES <1: note = Pent-4-ynoyl
  MOD_RES 3: note = HMSiR
SSCQLL

SEQ ID NO: 6 - protein, 6 aa, synthetic construct
  MOD_RES <1: note = Pent-4-ynoyl
  MOD_RES 3: note = HMSiR
  MOD_RES 2: note = phosphorylation
SSCQLL

SEQ ID NO: 7 - protein, 6 aa, synthetic construct
  MOD_RES <1: note = Pent-4-ynoyl
  MOD_RES 3: note = HMSiR
  MOD_RES 1: note = phosphorylation
SSCQLL

SEQ ID NO: 8 - protein, 16 aa, synthetic construct
  MOD_RES <1: note = Pent-4-ynoyl
  MOD_RES 10: note = HMSiR
GCWIAGSRGCGFVTRT

SEQ ID NO: 9 - protein, 16 aa, synthetic construct
  MOD_RES <1: note = Pent-4-ynoyl
  MOD_RES 3: note = HMSiR
  SITE 4: note = D-Isoleucine
GCWIAGSRGCGFVTRT

SEQ ID NO: 10 - protein, 16 aa, synthetic construct
  MOD_RES <1: note = Pent-4-ynoyl
  MOD_RES 3: note = HMSiR
  SITE 4: note = D-Isoleucine
  SITE 13: note = D-Valine
GCWIAGSRGCGFVTRT